European Patent Specification EP 3 856 767 B1, published March 27, 2024. Title: FORMULATIONS OF GLUCAGON-LIKE-PEPTIDE-2 (GLP-2) ANALOGUES. Applicant: ZEALAND PHARMA A/S. Application EP 18197750.5. The sequence listing filed with the application follows.

SEQUENCE LISTING (11 sequences)

SEQ ID NO: 1 - protein, 39 aa, Artificial Sequence
  Synthetic peptide sequence
HGEGTFSSELATILDALAARDFIAWLIATKITDKKKKKK

SEQ ID NO: 2 - protein, 36 aa, Artificial Sequence
  Synthetic peptide sequence
HGEGTFSSELATILDALAARDFIAWLIATKITDKKK

SEQ ID NO: 3 - protein, 35 aa, Artificial Sequence
  Synthetic peptide sequence
HGEGTFSSELATILDALAARDFIAWLIATKITDKK

SEQ ID NO: 4 - protein, 34 aa, Artificial Sequence
  Synthetic peptide sequence
HGEGTFSSELATILDALAARDFIAWLIATKITDK

SEQ ID NO: 5 - protein, 33 aa, Artificial Sequence
  Synthetic peptide sequence
HGEGTFSSELATILDALAARDFIAWLIATKITD

SEQ ID NO: 6 - protein, 33 aa, Artificial Sequence; identical to SEQ ID NO: 5
  Synthetic peptide sequence

SEQ ID NO: 7 - protein, 39 aa, Artificial Sequence
  Synthetic peptide sequence
HGEGSFSSELSTILDALAARDFIAWLIATKITDKKKKKK

SEQ ID NO: 8 - protein, 33 aa, Artificial Sequence
  Synthetic peptide sequence
HGEGSFSSELSTILDALAARDFIAWLIATKITD

SEQ ID NO: 9 - protein, 34 aa, Artificial Sequence
  Synthetic peptide sequence
HGEGSFSSELSTILDALAARDFIAWLIATKITDK

SEQ ID NO: 10 - protein, 33 aa, Homo sapiens
HADGSFSDEMNTILDNLAARDFINWLIQTKITD

SEQ ID NO: 11 - protein, 33 aa, Artificial Sequence
  Synthetic peptide sequence
  MISC_FEATURE (5)..(5): Xaa = Ser or Thr
  MISC_FEATURE (11)..(11): Xaa = Ala or Ser
HGEGXFSSELXTILDALAARDFIAWLIATKITD